European Patent Application EP 4 292 592 A1, published December 20, 2023. Title: Compositon for Controlling Sugar Containing Atypical PKC Activator. Applicant: Yonsei University Industry Foundation. The sequence listing filed with the application follows.

SEQUENCE LISTING (4 sequences)

SEQ ID NO: 1 - RNA, 25 nt, Artificial Sequence
  PKC siRNA
gggaugucagagagcaugccuucuu

SEQ ID NO: 2 - RNA, 19 nt, Artificial Sequence
  PKC siRNA
cucacaguacuuccucugu

SEQ ID NO: 3 - RNA, 25 nt, Artificial Sequence
  PKC siRNA
gcugagaucuguaucgcucucaacu

SEQ ID NO: 4 - RNA, 25 nt, Artificial Sequence
  PKC siRNA
ggacaauguacugcuagacucugaa